European Patent Application EP 4 155 317 A1, published March 29, 2023. Title: ANTI EOTAXIN-2 ANTIBODIES THAT RECOGNIZE ADDITIONAL CCR3-BINDING CHEMOKINES. Applicant: Chemomab Ltd. The sequence listing filed with the application follows.

SEQUENCE LISTING (19 sequences)

SEQ ID NO: 1 - DNA, 360 bp, Homo sapiens
cagatccaattggtgcagtctggacctgagctgaagaagcctggagcctcagtcaaggtctcctgcagggcttctgggtatcccttcacaaactctggaatgaactgggtaaagcaggctccaggaaagggtttaaagtggatgggctggatcaacacctacaatggagagccaacatatactgatgacttcaagggacggtttgccttctctttggaaacctctgccagcactgcctatttgcagatcaacaacctcagaaatgaggacacggctacatatttctgtgcaagtcattcctacggtagtagctacgctatggacaactggggtcaaggaacctcagtcaccgtctcctca

SEQ ID NO: 2 - DNA, 333 bp, Homo sapiens
gacattgtgctgacccaatctccagactctttggctgtgtctctaggggagagggccaccatcaactgcaaggccagccaaagtgttgattatgatggtgatagttatatgaactggtaccaacagaaaccaggacagccacccaaactcctcatctatgttgcatccaatctaaaatctggcatcccagccaggtttagtggcagtgggtctgggacagacttcaccctcaccatcagcagcctgcagcctgaggattttgcaacctattactgtcagcaaagtaatgaggaaccgtggacgttcggtggaggcaccaaggtggaaatcaaa

SEQ ID NO: 3 - protein, 120 aa, Homo sapiens
QIQLVQSGPELKKPGASVKVSCRASGYPFTNSGMNWVKQAPGKGLKWMGWINTYNGEPTYTDDFKGRFAFSLETSASTAYLQINNLRNEDTATYFCASHSYGSSYAMDNWGQGTSVTVSS

SEQ ID NO: 4 - protein, 111 aa, Homo sapiens
DIVLTQSPDSLAVSLGERATINCKASQSVDYDGDSYMNWYQQKPGQPPKLLIYVASNLKSGIPARFSGSGSGTDFTLTISSLQPEDFATYYCQQSNEEPWTFGGGTKVEIK

SEQ ID NO: 5 - protein, 5 aa, Homo sapiens
NSGMN

SEQ ID NO: 6 - protein, 17 aa, Homo sapiens
WINTYNGEPTYTDDFKG

SEQ ID NO: 7 - protein, 11 aa, Homo sapiens
HSYGSSYAMDN

SEQ ID NO: 8 - protein, 15 aa, Homo sapiens
KASQSVDYDGDSYMN

SEQ ID NO: 9 - protein, 7 aa, Homo sapiens
VASNLKS

SEQ ID NO: 10 - protein, 9 aa, Homo sapiens
QQSNEEPWT

SEQ ID NO: 11 - protein, 93 aa, Homo sapiens
VVIPSPCCMFFVSKRIPENRVVSYQLSSRSTCLKAGVIFTTKKGQQFCGDPKQEWVQRYMKNLDAKQKKASPRARAVAVKGPVQRYPGNQTTC

SEQ ID NO: 12 - protein, 74 aa, Homo sapiens
GPASVPTTCCFNLANRKIPLQRLESYRRITSGKCPQKAVIFKTKLAKDICADPKKKWVQDSMKYLDQKSPTPKP

SEQ ID NO: 13 - protein, 68 aa, Homo sapiens
SPYSSDTTPCCFAYIARPLPRAHIKEYFYTSGKCSNPAVVFVTRKNRQVCANPEKKWVREYINSLEMS

SEQ ID NO: 14 - protein, 76 aa, Homo sapiens
QPVGINTSTTCCYRFINKKIPKQRLESYRRTTSSHCPREAVIFKTKLDKEICADPTQKWVQDFMKHLDKKTQTPKL

SEQ ID NO: 15 - protein, 10 aa, Homo sapiens
CMFFVSKRIP

SEQ ID NO: 16 - protein, 14 aa, Homo sapiens
CFNLANRKIPLQRL

SEQ ID NO: 17 - protein, 17 aa, Homo sapiens
AYIARPLPRAHIKEYFY

SEQ ID NO: 18 - protein, 10 aa, Homo sapiens
CCYRFINKKI

SEQ ID NO: 19 - protein, 9 aa, Homo sapiens
SYRRTTSSH